European Patent Specification EP 3 583 203 B1, published November 1, 2023. Title: DONOR REPAIR TEMPLATES MULTIPLEX GENOME EDITING. Applicant: bluebird bio, Inc. Lee, Baeckseung Astrakhan, Alexander. The sequence listing filed with the application follows.

SEQUENCE LISTING (39 sequences)

SEQ ID NO: 1 - DNA, 7317 bp, Artificial Sequence
  Synthesized sequence pBW1411
cagctgcgcgctcgctcgctcactgaggccgcccgggcaaagcccgggcgtcgggcgacctttggtcgcccggcctcagtgagcgagcgagcgcgcagagagggagtggccaactccatcactaggggttccttgtagttaatgattaacccgccatgctacttatctacgtaaggctgttgcaggcatcacacggtggaaagatctggaactgtggccatggtgtgaggccatccacaaggtggaagctttgagggggagccgattagccatggacagttgtcattcagtagggtcacctgtgccccagcgaagggggatgggccgggaaggcagaggccaggcacctgcccccagcaggggcagaggctgtgggcagccgggaggctcccagaggctccgacagaatgggagtggggttgagcccacccctcactgcagcccaggaacctgagcccagagggggccacccaccttccccaggcagggaggcccggcccccagggagatgggggggatgggggaggagaagggcctgcccccacccggcagcctcaggaggggcagctcgggcgggatatggaaagaggccacagcagtgagcagagacacagaggaggaaggggccctgagctggggagacccccacggggtagggcgtgggggccacgggcccacctcctccccatctcctctgtctccctgtctctgtctctctctccctcccccaccctctccccagtcctaccccctcctcacccctcctcccccagcactgcctctgtcactctcgcccacgtggatgtggaggaagagggggcgggagcaaggggcgggcaccctcccttcaacctgacctgggacagtttcccttccgctcacctccgcctgagcagtggagaaggcggcactctggtggggctgctccaaatcatggcctcttggccaagattgatagcttgtgcctgtccctgagtcccagtccatcacgagcagctggtttctaagatgctatttcccgtataaagcatgagaccgtgacttgccagccccacagagccccgcccttgtccatcactggcatctggactccagcctgggttggggcaaagagggaaatgagatcatgtcctaaccctgatcctcttgtcccacagatatccagaaccctgaccctgccgtgtaccagctgagagactctaaatccagtgacaagtctgtctgcctatcgcgtgaacagagaaacaggagaatatgggccaaacaggatatctgtggtaagcagttcctgccccggctcagggccaagaacagttggaacagcagaatatgggccaaacaggatatctgtggtaagcagttcctgccccggctcagggccaagaacagatggtccccagatgcggtcccgccctcagcagtttctagagaaccatcagatgtttccagggtgccccaaggacctgaaatgaccctgtgccttatttgaactaaccaatcagttcgcttctcgcttctgttcgcgcgcttctgctccccgagctctatataagcagagctcgtttagtgaaccgtcagatcgcctggagacgccatccacgctgttttgacttccatagaaggatctcgaggccaccatggtgagcaagggcgaggagctgttcaccggggtggtgcccatcctggtcgagctggacggcgacgtaaacggccacaagttcagcgtgtccggcgagggcgagggcgatgccacctacggcaagctgaccctgaagttcatctgcaccaccggcaagctgcccgtgccctggcccaccctcgtgaccaccctgacctacggcgtgcagtgcttcagccgctaccccgaccacatgaagcagcacgacttcttcaagtccgccatgcccgaaggctacgtccaggagcgcaccatcttcttcaaggacgacggcaactacaagacccgcgccgaggtgaagttcgagggcgacaccctggtgaaccgcatcgagctgaagggcatcgacttcaaggaggacggcaacatcctggggcacaagctggagtacaactacaacagccacaacgtctatatcatggccgacaagcagaagaacggcatcaaggtgaacttcaagatccgccacaacatcgaggacggcagcgtgcagctcgccgaccactaccagcagaacacccccatcggcgacggccccgtgctgctgcccgacaaccactacctgagcacccagtccgccctgagcaaagaccccaacgagaagcgcgatcacatggtcctgctggagttcgtgaccgccgccgggatcactctcggcatggacgagctgtacaagtaagcggccgcgctttatttgtgaaatttgtgatgctattgctttatttgtaaccattataagctgcaataaacaagttaacaacaacaattgcattcattttatgtttcaggttcagggggagatgtgggaggttttttaaagcctctttgattctcaaacaaatgtgtcacaaagtaaggattctgatgtgtatatcacagacaaaactgtgctagacatgaggtctatggacttcaagagcaacagtgctgtggcctggagcaacaaatctgactttgcatgtgcaaacgccttcaacaacagcattattccagaagacaccttcttccccagcccaggtaagggcagctttggtgccttcgcaggctgtttccttgcttcaggaatggccaggttctgcccagagctctggtcaatgatgtctaaaactcctctgattggtggtaccggttctgggcggtgctacaactgggctggcggccaggatggttcttaggtaggtggggtcggcggtcaggtgtcccagagccaggggtctggagggaccttccaccctcagtccctggcaggtcggggggtgctgaggcgggcctggccctggcagcccaggggtcccggagcgaggggtctggagggacctttcactctcagtccctggcaggtcggggggtgctgtggcaggcccagccttggcccccagctctgccccttaccctgagctgtgtggctttgggcagctcgaactcctgggttcctctctgggccccaactcctcccctggcccaagtcccctctttgctcctgggcaggcaggacctctgtcccctctcagccggtccttggggctgcgtgtttctgtagaatgacgggtcaggctggccagaaccccaaaccttggccgtggggagtctgcgtggcggctctgccttgcccaggcatccttggtcctcactcgagttttcctaaggatgggatgagccccatgtgggactaaccttggctttacgacgtcaaagtttagatgagctggtgatatttttctcattatatccaaagtgtacctgttcgagtgaggacagttcttctgtctccaggatccctcctgggtggggattgtgcccgcctgggtctctgcccagattccagggctctccccgagccctgttcagaccatccgtgggggaggccttggcctcactcttacgtagataagtagcatggcgggttaatcattaactacaaggaacccctagtgatggagttggccactccctctctgcgcgctcgctcgctcactgaggccgggcgaccaaaggtcgcccgacgcccgggctttgcccgggcggcctcagtgagcgagcgagcgcgccagctggcgtaatagcgaagaggcccgcaccgatcgcccttcccaacagttgcgcagcctgaatggcgaatggcgattccgttgcaatggctggcggtaatattgttctggatattaccagcaaggccgatagtttgagttcttctactcaggcaagtgatgttattactaatcaaagaagtattgcgacaacggttaatttgcgtgatggacagactcttttactcggtggcctcactgattataaaaacacttctcaggattctggcgtaccgttcctgtctaaaatccctttaatcggcctcctgtttagctcccgctctgattctaacgaggaaagcacgttatacgtgctcgtcaaagcaaccatagtacgcgccctgtagcggcgcattaagcgcggcgggtgtggtggttacgcgcagcgtgaccgctacacttgccagcgccctagcgcccgctcctttcgctttcttcccttcctttctcgccacgttcgccggctttccccgtcaagctctaaatcgggggctccctttagggttccgatttagtgctttacggcacctcgaccccaaaaaacttgattagggtgatggttcacgtagtgggccatcgccctgatagacggtttttcgccctttgacgttggagtccacgttctttaatagtggactcttgttccaaactggaacaacactcaaccctatctcggtctattcttttgatttataagggattttgccgatttcggcctattggttaaaaaatgagctgatttaacaaaaatttaacgcgaattttaacaaaatattaacgtttacaatttaaatatttgcttatacaatcttcctgtttttggggcttttctgattatcaaccggggtacatatgattgacatgctagttttacgattaccgttcatcgattctcttgtttgctccagactctcaggcaatgacctgatagcctttgtagagacctctcaaaaatagctaccctctccggcatgaatttatcagctagaacggttgaatatcatattgatggtgatttgactgtctccggcctttctcacccgtttgaatctttacctacacattactcaggcattgcatttaaaatatatgagggttctaaaaatttttatccttgcgttgaaataaaggcttctcccgcaaaagtattacagggtcataatgtttttggtacaaccgatttagctttatgctctgaggctttattgcttaattttgctaattctttgccttgcctgtatgatttattggatgttggaatcgcctgatgcggtattttctccttacgcatctgtgcggtatttcacaccgcatatggtgcactctcagtacaatctgctctgatgccgcatagttaagccagccccgacacccgccaacacccgctgacgcgccctgacgggcttgtctgctcccggcatccgcttacagacaagctgtgaccgtctccgggagctgcatgtgtcagaggttttcaccgtcatcaccgaaacgcgcgagacgaaagggcctcgtgatacgcctatttttataggttaatgtcatgataataatggtttcttagacgtcaggtggcacttttcggggaaatgtgcgcggaacccctatttgtttatttttctaaatacattcaaatatgtatccgctcatgagacaataaccctgataaatgcttcaataatattgaaaaaggaagagtatgagtattcaacatttccgtgtcgcccttattcccttttttgcggcattttgccttcctgtttttgctcacccagaaacgctggtgaaagtaaaagatgctgaagatcagttgggtgcacgagtgggttacatcgaactggatctcaacagcggtaagatccttgagagttttcgccccgaagaacgttttccaatgatgagcacttttaaagttctgctatgtggcgcggtattatcccgtattgacgccgggcaagagcaactcggtcgccgcatacactattctcagaatgacttggttgagtactcaccagtcacagaaaagcatcttacggatggcatgacagtaagagaattatgcagtgctgccataaccatgagtgataacactgcggccaacttacttctgacaacgatcggaggaccgaaggagctaaccgcttttttgcacaacatgggggatcatgtaactcgccttgatcgttgggaaccggagctgaatgaagccataccaaacgacgagcgtgacaccacgatgcctgtagcaatggcaacaacgttgcgcaaactattaactggcgaactacttactctagcttcccggcaacaattaatagactggatggaggcggataaagttgcaggaccacttctgcgctcggcccttccggctggctggtttattgctgataaatctggagccggtgagcgtgggtctcgcggtatcattgcagcactggggccagatggtaagccctcccgtatcgtagttatctacacgacggggagtcaggcaactatggatgaacgaaatagacagatcgctgagataggtgcctcactgattaagcattggtaactgtcagaccaagtttactcatatatactttagattgatttaaaacttcatttttaatttaaaaggatctaggtgaagatcctttttgataatctcatgaccaaaatcccttaacgtgagttttcgttccactgagcgtcagaccccgtagaaaagatcaaaggatcttcttgagatcctttttttctgcgcgtaatctgctgcttgcaaacaaaaaaaccaccgctaccagcggtggtttgtttgccggatcaagagctaccaactctttttccgaaggtaactggcttcagcagagcgcagataccaaatactgtccttctagtgtagccgtagttaggccaccacttcaagaactctgtagcaccgcctacatacctcgctctgctaatcctgttaccagtggctgctgccagtggcgataagtcgtgtcttaccgggttggactcaagacgatagttaccggataaggcgcagcggtcgggctgaacggggggttcgtgcacacagcccagcttggagcgaacgacctacaccgaactgagatacctacagcgtgagctatgagaaagcgccacgcttcccgaagggagaaaggcggacaggtatccggtaagcggcagggtcggaacaggagagcgcacgagggagcttccagggggaaacgcctggtatctttatagtcctgtcgggtttcgccacctctgacttgagcgtcgatttttgtgatgctcgtcaggggggcggagcctatggaaaaacgccagcaacgcggcctttttacggttcctggccttttgctggccttttgctcacatgttctttcctgcgttatcccctgattctgtggataaccgtattaccgcctttgagtgagctgataccgctcgccgcagccgaacgaccgagcgcagcgagtcagtgagcgaggaagcggaagagcgcccaatacgcaaaccgcctctccccgcgcgttggccgattcattaatg

SEQ ID NO: 2 - DNA, 7413 bp, Artificial Sequence
  Synthesized sequence pBW1490
cagctgcgcgctcgctcgctcactgaggccgcccgggcaaagcccgggcgtcgggcgacctttggtcgcccggcctcagtgagcgagcgagcgcgcagagagggagtggccaactccatcactaggggttccttgtagttaatgattaacccgccatgctacttatctacgtaatgggggaggagaagggcctgcccccacccggcagcctcaggaggggcagctcgggcgggatatggaaagaggccacagcagtgagcagagacacagaggaggaaggggccctgagctggggagacccccacggggtagggcgtgggggccacgggcccacctcctccccatctcctctgtctccctgtctctgtctctctctccctcccccaccctctccccagtcctaccccctcctcacccctcctcccccagcactgcctctgtcactctcgcccacgtggatgtggaggaagagggggcgggagcaaggggcgggcaccctcccttcaacctgacctgggacagtttcccttccgctcacctccgcctgagcagtggagaaggcggcactctggtggggctgctccaaatcatggcctcttggccaagattgatagcttgtgcctgtccctgagtcccagtccatcacgagcagctggtttctaagatgctatttcccgtataaagcatgagaccgtgacttgccagccccacagagccccgcccttgtccatcactggcatctggactccagcctgggttggggcaaagagggaaatgagatcatgtcctaaccctgatcctcttgtcccacagatatccagaaccctgaccctgccgtgtaccagctgagagactctaaatccagtgacaagtctgtctgcctatacgcgtaatgaaagaccccacctgtaggtttggcaagctaggatcaaggttaggaacagagagacagcagaatatgggccaaacaggatatctgtggtaagcagttcctgccccggctcagggccaagaacagttggaacagcagaatatgggccaaacaggatatctgtggtaagcagttcctgccccggctcagggccaagaacagatggtccccagatgcggtcccgccctcagcagtttctagagaaccatcagatgtttccagggtgccccaaggacctgaaatgaccctgtgccttatttgaactaaccaatcagttcgcttctcgcttctgttcgcgcgcttctgctccccgagctcaataaaagagcccacaacccctcactcggcgcgattcacctgcgcgtctacgccaccatggcactccccgtcaccgcccttctcttgcccctcgccctgctgctgcatgctgccaggcccgacattgtgctcactcagtcacctcccagcctggccatgagcctgggaaaaagggccaccatctcctgtagagccagtgagtccgtcacaatcttggggagccatcttattcactggtatcagcagaagcccgggcagcctccaacccttcttattcagctcgcgtcaaacgtccagacgggtgtacctgccagattttctggtagcgggtcccgcactgattttacactgaccatagatccagtggaagaagacgatgtggccgtgtattattgtctgcagagcagaacgattcctcgcacatttggtgggggtactaagctggagattaagggaagcacgtccggctcagggaagccgggctccggcgagggaagcacgaaggggcaaattcagctggtccagagcggacctgagctgaaaaaacccggcgagactgttaagatcagttgtaaagcatctggctataccttcaccgactacagcataaattgggtgaaacgggcccctggaaagggcctcaaatggatgggttggatcaataccgaaactagggagcctgcttatgcatatgacttccgcgggagattcgccttttcactcgagacatctgcctctactgcttacctccaaataaacaacctcaagtatgaagatacagccacttacttttgcgccctcgactatagttacgccatggactactggggacagggaacctccgttaccgtcagttccgcggccgcaaccacaacacctgctccaaggccccccacacccgctccaactatagccagccaaccattgagcctcagacctgaagcttgcaggcccgcagcaggaggcgccgtccatacgcgaggcctggacttcgcgtgtgatatttatatttgggcccctttggccggaacatgtggggtgttgcttctctcccttgtgatcactctgtattgtaagcgcgggagaaagaagctcctgtacatcttcaagcagccttttatgcgacctgtgcaaaccactcaggaagaagatgggtgttcatgccgcttccccgaggaggaagaaggagggtgtgaactgagggtgaaattttctagaagcgccgatgctcccgcatatcagcagggtcagaatcagctctacaatgaattgaatctcggcaggcgagaagagtacgatgttctggacaagagacggggcagggatcccgagatggggggaaagccccggagaaaaaatcctcaggaggggttgtacaatgagctgcagaaggacaagatggctgaagcctatagcgagatcggaatgaaaggcgaaagacgcagaggcaaggggcatgacggtctgtaccagggtctctctacagccaccaaggacacttatgatgcgttgcatatgcaagccttgccaccccgctaagcggccgcgctttatttgtgaaatttgtgatgctattgctttatttgtaaccattataagctgcaataaacaagttaacaacaacaattgcattcattttatgtttcaggttcagggggagatgtgggaggttttttaaagctcaccggttttgattctcaaacaaatgtgtcacaaagtaaggattctgatgtgtatatcacagacaaaactgtgctagacatgaggtctatggacttcaagagcaacagtgctgtggcctggagcaacaaatctgactttgcatgtgcaaacgccttcaacaacagcattattccagaagacaccttcttccccagcccaggtaagggcagctttggtgccttcgcaggctgtttccttgcttcaggaatggccaggttctgcccagagctctggtcaatgatgtctaaaactcctctgattggtggtaccggttctgggcggtgctacaactgggctggcggccaggatggttcttaggtaggtggggtcggcggtcaggtgtcccagagccaggggtctggagggaccttccaccctcagtccctggcaggtcggggggtgctgaggcgggcctggccctggcagcccaggggtcccggagcgaggggtctggagggacctttcactctcagtccctggcaggtcggggggtgctgtggcaggcccagccttggcccccagctctgccccttaccctgagctgtgtggctttgggcagctcgaactcctgggttcctctctgggccccaactcctcccctggcccaagtcccctctttgctcctgggcaggcaggacctctgtcccctctcagccggtccttggggctgcgtgtttctgtagtacgtagataagtagcatggcgggttaatcattaactacaaggaacccctagtgatggagttggccactccctctctgcgcgctcgctcgctcactgaggccgggcgaccaaaggtcgcccgacgcccgggctttgcccgggcggcctcagtgagcgagcgagcgcgccagctggcgtaatagcgaagaggcccgcaccgatcgcccttcccaacagttgcgcagcctgaatggcgaatggcgattccgttgcaatggctggcggtaatattgttctggatattaccagcaaggccgatagtttgagttcttctactcaggcaagtgatgttattactaatcaaagaagtattgcgacaacggttaatttgcgtgatggacagactcttttactcggtggcctcactgattataaaaacacttctcaggattctggcgtaccgttcctgtctaaaatccctttaatcggcctcctgtttagctcccgctctgattctaacgaggaaagcacgttatacgtgctcgtcaaagcaaccatagtacgcgccctgtagcggcgcattaagcgcggcgggtgtggtggttacgcgcagcgtgaccgctacacttgccagcgccctagcgcccgctcctttcgctttcttcccttcctttctcgccacgttcgccggctttccccgtcaagctctaaatcgggggctccctttagggttccgatttagtgctttacggcacctcgaccccaaaaaacttgattagggtgatggttcacgtagtgggccatcgccctgatagacggtttttcgccctttgacgttggagtccacgttctttaatagtggactcttgttccaaactggaacaacactcaaccctatctcggtctattcttttgatttataagggattttgccgatttcggcctattggttaaaaaatgagctgatttaacaaaaatttaacgcgaattttaacaaaatattaacgtttacaatttaaatatttgcttatacaatcttcctgtttttggggcttttctgattatcaaccggggtacatatgattgacatgctagttttacgattaccgttcatcgattctcttgtttgctccagactctcaggcaatgacctgatagcctttgtagagacctctcaaaaatagctaccctctccggcatgaatttatcagctagaacggttgaatatcatattgatggtgatttgactgtctccggcctttctcacccgtttgaatctttacctacacattactcaggcattgcatttaaaatatatgagggttctaaaaatttttatccttgcgttgaaataaaggcttctcccgcaaaagtattacagggtcataatgtttttggtacaaccgatttagctttatgctctgaggctttattgcttaattttgctaattctttgccttgcctgtatgatttattggatgttggaatcgcctgatgcggtattttctccttacgcatctgtgcggtatttcacaccgcatatggtgcactctcagtacaatctgctctgatgccgcatagttaagccagccccgacacccgccaacacccgctgacgcgccctgacgggcttgtctgctcccggcatccgcttacagacaagctgtgaccgtctccgggagctgcatgtgtcagaggttttcaccgtcatcaccgaaacgcgcgagacgaaagggcctcgtgatacgcctatttttataggttaatgtcatgataataatggtttcttagacgtcaggtggcacttttcggggaaatgtgcgcggaacccctatttgtttatttttctaaatacattcaaatatgtatccgctcatgagacaataaccctgataaatgcttcaataatattgaaaaaggaagagtatgagtattcaacatttccgtgtcgcccttattcccttttttgcggcattttgccttcctgtttttgctcacccagaaacgctggtgaaagtaaaagatgctgaagatcagttgggtgcacgagtgggttacatcgaactggatctcaacagcggtaagatccttgagagttttcgccccgaagaacgttttccaatgatgagcacttttaaagttctgctatgtggcgcggtattatcccgtattgacgccgggcaagagcaactcggtcgccgcatacactattctcagaatgacttggttgagtactcaccagtcacagaaaagcatcttacggatggcatgacagtaagagaattatgcagtgctgccataaccatgagtgataacactgcggccaacttacttctgacaacgatcggaggaccgaaggagctaaccgcttttttgcacaacatgggggatcatgtaactcgccttgatcgttgggaaccggagctgaatgaagccataccaaacgacgagcgtgacaccacgatgcctgtagcaatggcaacaacgttgcgcaaactattaactggcgaactacttactctagcttcccggcaacaattaatagactggatggaggcggataaagttgcaggaccacttctgcgctcggcccttccggctggctggtttattgctgataaatctggagccggtgagcgtgggtctcgcggtatcattgcagcactggggccagatggtaagccctcccgtatcgtagttatctacacgacggggagtcaggcaactatggatgaacgaaatagacagatcgctgagataggtgcctcactgattaagcattggtaactgtcagaccaagtttactcatatatactttagattgatttaaaacttcatttttaatttaaaaggatctaggtgaagatcctttttgataatctcatgaccaaaatcccttaacgtgagttttcgttccactgagcgtcagaccccgtagaaaagatcaaaggatcttcttgagatcctttttttctgcgcgtaatctgctgcttgcaaacaaaaaaaccaccgctaccagcggtggtttgtttgccggatcaagagctaccaactctttttccgaaggtaactggcttcagcagagcgcagataccaaatactgtccttctagtgtagccgtagttaggccaccacttcaagaactctgtagcaccgcctacatacctcgctctgctaatcctgttaccagtggctgctgccagtggcgataagtcgtgtcttaccgggttggactcaagacgatagttaccggataaggcgcagcggtcgggctgaacggggggttcgtgcacacagcccagcttggagcgaacgacctacaccgaactgagatacctacagcgtgagctatgagaaagcgccacgcttcccgaagggagaaaggcggacaggtatccggtaagcggcagggtcggaacaggagagcgcacgagggagcttccagggggaaacgcctggtatctttatagtcctgtcgggtttcgccacctctgacttgagcgtcgatttttgtgatgctcgtcaggggggcggagcctatggaaaaacgccagcaacgcggcctttttacggttcctggccttttgctggccttttgctcacatgttctttcctgcgttatcccctgattctgtggataaccgtattaccgcctttgagtgagctgataccgctcgccgcagccgaacgaccgagcgcagcgagtcagtgagcgaggaagcggaagagcgcccaatacgcaaaccgcctctccccgcgcgttggccgattcattaatg

SEQ ID NO: 3 - protein, 3 aa, Artificial Sequence
  Exemplary linker sequence
GGG

SEQ ID NO: 4 - protein, 5 aa, Artificial Sequence
  Exemplary linker sequence
DGGGS

SEQ ID NO: 5 - protein, 5 aa, Artificial Sequence
  Exemplary linker sequence
TGEKP

SEQ ID NO: 6 - protein, 4 aa, Artificial Sequence
  Exemplary linker sequence
GGRR

SEQ ID NO: 7 - protein, 5 aa, Artificial Sequence
  Exemplary linker sequence
GGGGS

SEQ ID NO: 8 - protein, 14 aa, Artificial Sequence
  Exemplary linker sequence
EGKSSGSGSESKVD

SEQ ID NO: 9 - protein, 18 aa, Artificial Sequence
  Exemplary linker sequence
KESGSVSSEQLAQFRSLD

SEQ ID NO: 10 - protein, 8 aa, Artificial Sequence
  Exemplary linker sequence
GGRRGGGS

SEQ ID NO: 11 - protein, 9 aa, Artificial Sequence
  Exemplary linker sequence
LRQRDGERP

SEQ ID NO: 12 - protein, 12 aa, Artificial Sequence
  Exemplary linker sequence
LRQKDGGGSERP

SEQ ID NO: 13 - protein, 16 aa, Artificial Sequence
  Exemplary linker sequence
LRQKDGGGSGGGSERP

SEQ ID NO: 14 - protein, 7 aa, Artificial Sequence
  Cleavage sequence by TEV protease
  misc_feature (2)..(3): Xaa is any amino acid
  misc_feature (5)..(5): Xaa is any amino acid
  MISC_FEATURE (7)..(7): Xaa = Gly or Ser
EXXYXQX

SEQ ID NO: 15 - protein, 7 aa, Artificial Sequence
  Cleavage sequence by TEV protease
ENLYFQG

SEQ ID NO: 16 - protein, 7 aa, Artificial Sequence
  Cleavage sequence by TEV protease
ENLYFQS

SEQ ID NO: 17 - protein, 22 aa, Artificial Sequence
  Self-cleaving polypeptide comprising 2A site
GSGATNFSLLKQAGDVEENPGP

SEQ ID NO: 18 - protein, 19 aa, Artificial Sequence
  Self-cleaving polypeptide comprising 2A site
ATNFSLLKQAGDVEENPGP

SEQ ID NO: 19 - protein, 14 aa, Artificial Sequence
  Self-cleaving polypeptide comprising 2A site
LLKQAGDVEENPGP

SEQ ID NO: 20 - protein, 21 aa, Artificial Sequence
  Self-cleaving polypeptide comprising 2A site
GSGEGRGSLLTCGDVEENPGP

SEQ ID NO: 21 - protein, 18 aa, Artificial Sequence
  Self-cleaving polypeptide comprising 2A site
EGRGSLLTCGDVEENPGP

SEQ ID NO: 22 - protein, 13 aa, Artificial Sequence
  Self-cleaving polypeptide comprising 2A site
LLTCGDVEENPGP

SEQ ID NO: 23 - protein, 23 aa, Artificial Sequence
  Self-cleaving polypeptide comprising 2A site
GSGQCTNYALLKLAGDVESNPGP

SEQ ID NO: 24 - protein, 20 aa, Artificial Sequence
  Self-cleaving polypeptide comprising 2A site
QCTNYALLKLAGDVESNPGP

SEQ ID NO: 25 - protein, 14 aa, Artificial Sequence
  Self-cleaving polypeptide comprising 2A site
LLKLAGDVESNPGP

SEQ ID NO: 26 - protein, 25 aa, Artificial Sequence
  Self-cleaving polypeptide comprising 2A site
GSGVKQTLNFDLLKLAGDVESNPGP

SEQ ID NO: 27 - protein, 22 aa, Artificial Sequence
  Self-cleaving polypeptide comprising 2A site
VKQTLNFDLLKLAGDVESNPGP

SEQ ID NO: 28 - protein, 14 aa, Artificial Sequence
  Self-cleaving polypeptide comprising 2A site
LLKLAGDVESNPGP

SEQ ID NO: 29 - protein, 19 aa, Artificial Sequence
  Self-cleaving polypeptide comprising 2A site
LLNFDLLKLAGDVESNPGP

SEQ ID NO: 30 - protein, 19 aa, Artificial Sequence
  Self-cleaving polypeptide comprising 2A site
TLNFDLLKLAGDVESNPGP

SEQ ID NO: 31 - protein, 14 aa, Artificial Sequence
  Self-cleaving polypeptide comprising 2A site
LLKLAGDVESNPGP

SEQ ID NO: 32 - protein, 17 aa, Artificial Sequence
  Self-cleaving polypeptide comprising 2A site
NFDLLKLAGDVESNPGP

SEQ ID NO: 33 - protein, 20 aa, Artificial Sequence
  Self-cleaving polypeptide comprising 2A site
QLLNFDLLKLAGDVESNPGP

SEQ ID NO: 34 - protein, 24 aa, Artificial Sequence
  Self-cleaving polypeptide comprising 2A site
APVKQTLNFDLLKLAGDVESNPGP

SEQ ID NO: 35 - protein, 40 aa, Artificial Sequence
  Self-cleaving polypeptide comprising 2A site
VTELLYRMKRAETYCPRPLLAIHPTEARHKQKIVAPVKQT

SEQ ID NO: 36 - protein, 18 aa, Artificial Sequence
  Self-cleaving polypeptide comprising 2A site
LNFDLLKLAGDVESNPGP

SEQ ID NO: 37 - protein, 40 aa, Artificial Sequence
  Self-cleaving polypeptide comprising 2A site
LLAIHPTEARHKQKIVAPVKQTLNFDLLKLAGDVESNPGP

SEQ ID NO: 38 - protein, 33 aa, Artificial Sequence
  Self-cleaving polypeptide comprising 2A site
EARHKQKIVAPVKQTLNFDLLKLAGDVESNPGP

SEQ ID NO: 39 - DNA, 10 bp, Artificial Sequence
  Consensus Kozak sequence
gccrccatgg